European Patent Specification EP 3 775 053 B1, published September 6, 2023. Title: Fibrin-Specific Materials and Methods of Using Thereof. Applicant: NORTH CAROLINA STATE UNIVERSITY. Application EP19781458.5, based on PCT/US2019/025839. The sequence listing filed with the application follows.

SEQUENCE LISTING (3 sequences)

SEQ ID NO: 1 - protein, 144 aa, pyrrolysine
  misc_feature (3)..(3): pyrrolysine
  misc_feature (13)..(13): pyrrolysine
  misc_feature (82)..(82): pyrrolysine
  misc_feature (113)..(113): pyrrolysine
  misc_feature (126)..(126): pyrrolysine
QVXLLESGGGLVXPGGSLRLSCAASGDRFTHNDMGWWRQAPGKGLEWWSTIPTTDGSTYYADSVKGRFTISRDNSKSTLYLXMNSLRAEDTAVYYCATGYMWKAPAYWKYWGXGTLWTVSSAAAEXKLISEEDLNSAAHYTDIG

SEQ ID NO: 2 - protein, 142 aa, pyrrolysine
  misc_feature (3)..(3): pyrrolysine
  misc_feature (13)..(13): pyrrolysine
  misc_feature (39)..(39): pyrrolysine
  misc_feature (82)..(82): pyrrolysine
  misc_feature (111)..(111): pyrrolysine
  misc_feature (124)..(124): pyrrolysine
QVXLLESGGGLVXPGGSLRLSCAASGFSLNDKIMTWVRXAPGKGLEWVSSISGPNGSTYYADSVKGRFTISRDNSKNTLYLXMNSLRAEDTAVYYCAGCAAASSTMEYWGXGTLVTVSSAAAEXKLISEEDLNSAAHYTDIR

SEQ ID NO: 3 - protein, 147 aa, pyrrolysine
  misc_feature (3)..(3): pyrrolysine
  misc_feature (13)..(13): pyrrolysine
  misc_feature (39)..(39): pyrrolysine
  misc_feature (82)..(82): pyrrolysine
  misc_feature (108)..(108): pyrrolysine
  misc_feature (115)..(115): pyrrolysine
  misc_feature (128)..(128): pyrrolysine
QVXLLESGGGLVXPGGSLRLSCAASGWRITDDSMSWVRXAPGKGLEWVSSIEDNSGSTYYADSVKGRFTISRDNSKNTLYLXMNSLRAEDTAVYYCAGEGWDVLRRDXAVTSWGXGTLVTVSSAAAEXKLISEEDLINSAAHYTDMR